European Patent Specification EP 3 596 120 B1, published December 13, 2023. Title: Collagen Type XVIII Assay. Applicant: Nordic Bioscience A/S. The sequence listing filed with the application follows.

SEQUENCE LISTING (9 sequences)

SEQ ID NO: 1 - protein, 10 aa, Artificial Sequence
  Target N-terminal sequence
EPERISEEVG

SEQ ID NO: 2 - protein, 6 aa, Artificial Sequence
  Target sequence N-terminal
EPERIS

SEQ ID NO: 3 - protein, 11 aa, Artificial Sequence
  N-extended peptide
AEPERISEEVG

SEQ ID NO: 4 - protein, 9 aa, Artificial Sequence
  N-truncated peptide
PERISEEVG

SEQ ID NO: 5 - protein, 10 aa, Artificial Sequence
  C-terminal biotinylated peptide with optional linker between peptide and biotin
  SITE 10: C-terminus biotinylated with optional linker between C-terminus of peptide and biotin residue
EPERISEEVG

SEQ ID NO: 6 - protein, 10 aa, Artificial Sequence
  Calibration peptide
EPERISEEVG

SEQ ID NO: 7 - protein, 11 aa, Artificial Sequence
  Biotinylated coater peptide
  SITE 11: C-terminus biotinylated
EPERISEEVGK

SEQ ID NO: 8 - protein, 9 aa, Artificial Sequence
  nonsense peptide
EPQIDEKKK

SEQ ID NO: 9 - protein, 9 aa, Artificial Sequence
  nonsense peptide
CPERALERR